European Patent Specification EP 3 608 419 B1, published March 26, 2025. Title: BIOMARKER FOR USE IN TREATING ANEMIA. Applicant: Celgene Corporation. Application Divisional patent application based on EP 13848471.2. The sequence listing filed with the application follows.

SEQUENCE LISTING (53 sequences)

SEQ ID NO: 1 - protein, 513 aa, Homo sapiens
  human ActRIIA precursor polypeptide
MGAAAKLAFAVFLISCSSGAILGRSETQECLFFNANWEKDRTNQTGVEPCYGDKDKRRHCFATWKNISGSIEIVKQGCWLDDINCYDRTDCVEKKDSPEVYFCCCEGNMCNEKFSYFPEMEVTQPTSNPVTPKPPYYNILLYSLVPLMLIAGIVICAFWVYRHHKMAYPPVLVPTQDPGPPPPSPLLGLKPLQLLEVKARGRFGCVWKAQLLNEYVAVKIFPIQDKQSWQNEYEVYSLPGMKHENILQFIGAEKRGTSVDVDLWLITAFHEKGSLSDFLKANVVSWNELCHIAETMARGLAYLHEDIPGLKDGHKPAISHRDIKSKNVLLKNNLTACIADFGLALKFEAGKSAGDTHGQVGTRRYMAPEVLEGAINFQRDAFLRIDMYAMGLVLWELASRCTAADGPVDEYMLPFEEEIGQHPSLEDMQEVVVHKKKRPVLRDYWQKHAGMAMLCETIEECWDHDAEARLSAGCVGERITQMQRLTNIITTEDIVTVVTMVTNVDFPPKESSL

SEQ ID NO: 2 - protein, 115 aa, Homo sapiens
  human ActRIIA soluble (extracellular), processed polypeptide
ILGRSETQECLFFNANWEKDRTNQTGVEPCYGDKDKRRHCFATWKNISGSIEIVKQGCWLDDINCYDRTDCVEKKDSPEVYFCCCEGNMCNEKFSYFPEMEVTQPTSNPVTPKPP

SEQ ID NO: 3 - protein, 100 aa, Artificial Sequence
  human ActRIIA soluble (extracellular), processed polypeptide with the C-terminal 15 amino acids deleted
ILGRSETQECLFFNANWEKDRTNQTGVEPCYGDKDKRRHCFATWKNISGSIEIVKQGCWLDDINCYDRTDCVEKKDSPEVYFCCCEGNMCNEKFSYFPEM

SEQ ID NO: 4 - DNA, 1542 bp, Homo sapiens
  human ActRIIA precursor
atgggagctgctgcaaagttggcgtttgccgtctttcttatctcctgttcttcaggtgctatacttggtagatcagaaactcaggagtgtcttttctttaatgctaattgggaaaaagacagaaccaatcaaactggtgttgaaccgtgttatggtgacaaagataaacggcggcattgttttgctacctggaagaatatttctggttccattgaaatagtgaaacaaggttgttggctggatgatatcaactgctatgacaggactgattgtgtagaaaaaaaagacagccctgaagtatatttttgttgctgtgagggcaatatgtgtaatgaaaagttttcttattttccagagatggaagtcacacagcccacttcaaatccagttacacctaagccaccctattacaacatcctgctctattccttggtgccacttatgttaattgcggggattgtcatttgtgcattttgggtgtacaggcatcacaagatggcctaccctcctgtacttgttccaactcaagacccaggaccacccccaccttctccattactagggttgaaaccactgcagttattagaagtgaaagcaaggggaagatttggttgtgtctggaaagcccagttgcttaacgaatatgtggctgtcaaaatatttccaatacaggacaaacagtcatggcaaaatgaatacgaagtctacagtttgcctggaatgaagcatgagaacatattacagttcattggtgcagaaaaacgaggcaccagtgttgatgtggatctttggctgatcacagcatttcatgaaaagggttcactatcagactttcttaaggctaatgtggtctcttggaatgaactgtgtcatattgcagaaaccatggctagaggattggcatatttacatgaggatatacctggcctaaaagatggccacaaacctgccatatctcacagggacatcaaaagtaaaaatgtgctgttgaaaaacaacctgacagcttgcattgctgactttgggttggccttaaaatttgaggctggcaagtctgcaggcgatacccatggacaggttggtacccggaggtacatggctccagaggtattagagggtgctataaacttcgaaagggatgcatttttgaggatagatatgtatgccatgggattagtcctatgggaactggcttctcgctgtactgctgcagatggacctgtagatgaatacatgttgccatttgaggaggaaattggccagcatccatctcttgaagacatgcaggaagttgttgtgcataaaaaaaagaggcctgttttaagagattattggcagaaacatgctggaatggcaatgctctgtgaaaccattgaagaatgttgggatcacgacgcagaagccaggttatcagctggatgtgtaggtgaaagaattacccagatgcagagactaacaaatattattaccacagaggacattgtaacagtggtcacaatggtgacaaatgttgactttcctcccaaagaatctagtctatga

SEQ ID NO: 5 - DNA, 345 bp, Homo sapiens
  human ActRIIA soluble (extracellular) polypeptide
atacttggtagatcagaaactcaggagtgtcttttctttaatgctaattgggaaaaagacagaaccaatcaaactggtgttgaaccgtgttatggtgacaaagataaacggcggcattgttttgctacctggaagaatatttctggttccattgaaatagtgaaacaaggttgttggctggatgatatcaactgctatgacaggactgattgtgtagaaaaaaaagacagccctgaagtatatttttgttgctgtgagggcaatatgtgtaatgaaaagttttcttattttccagagatggaagtcacacagcccacttcaaatccagttacacctaagccaccc

SEQ ID NO: 6 - protein, 225 aa, Artificial Sequence
  Synthetic construct - fusion protein comprising a soluble extracellular domain of ActRIIA fused to an Fc domain
  MOD_RES (43)..(43): Asp or Ala
  MOD_RES (100)..(100): Lys or Ala
  MOD_RES (212)..(212): Asn or Ala
THTCPPCPAPELLGGPSVFLFPPKPKDTLMISRTPEVTCVVVXVSHEDPEVKFNWYVDGVEVHNAKTKPREEQYNSTYRVVSVLTVLHQDWLNGKEYKCXVSNKALPVPIEKTISKAKGQPREPQVYTLPPSREEMTKNQVSLTCLVKGFYPSDIAVEWESNGQPENNYKTTPPVLDSDGPFFLYSKLTVDKSRWQQGNVFSCSVMHEALHXHYTQKSLSLSPGK

SEQ ID NO: 7 - protein, 344 aa, Artificial Sequence
  Synthetic construct - Extracellular domain of human ActRIIA fused to a human Fc domain
ILGRSETQECLFFNANWEKDRTNQTGVEPCYGDKDKRRHCFATWKNISGSIEIVKQGCWLDDINCYDRTDCVEKKDSPEVYFCCCEGNMCNEKFSYFPEMEVTQPTSNPVTPKPPTGGGTHTCPPCPAPELLGGPSVFLFPPKPKDTLMISRTPEVTCVVVDVSHEDPEVKFNWYVDGVEVHNAKTKPREEQYNSTYRVVSVLTVLHQDWLNGKEYKCKVSNKALPVPIEKTISKAKGQPREPQVYTLPPSREEMTKNQVSLTCLVKGFYPSDIAVEWESNGQPENNYKTTPPVLDSDGSFFLYSKLTVDKSRWQQGNVFSCSVMHEALHNHYTQKSLSLSPGK

SEQ ID NO: 8 - protein, 21 aa, Apis mellifera
  Leader sequence of Honey bee mellitin
MKFLVNVALVFMVVYISYIYA

SEQ ID NO: 9 - protein, 22 aa, Unknown
  Leader sequence of Tissue Plasminogen Activator (TPA)
MDAMKRGLCCVLLLCGAVFVSP

SEQ ID NO: 10 - protein, 20 aa, Unknown
  Native ActRIIA leader
MGAAAKLAFAVFLISCSSGA

SEQ ID NO: 11 - protein, 9 aa, Artificial Sequence
  Synthetic construct - ActRIIA-hFc and ActRIIA-mFc N-terminal sequence
ILGRSETQE

SEQ ID NO: 12 - protein, 329 aa, Artificial Sequence
  Synthetic construct - ActRIIA-Fc Protein with deletion of the C-terminal 15 amino acids of the extracellular domain of ActRIIA
ILGRSETQECLFFNANWEKDRTNQTGVEPCYGDKDKRRHCFATWKNISGSIEIVKQGCWLDDINCYDRTDCVEKKDSPEVYFCCCEGNMCNEKFSYFPEMTGGGTHTCPPCPAPELLGGPSVFLFPPKPKDTLMISRTPEVTCVVVDVSHEDPEVKFNWYVDGVEVHNAKTKPREEQYNSTYRVVSVLTVLHQDWLNGKEYKCKVSNKALPVPIEKTISKAKGQPREPQVYTLPPSREEMTKNQVSLTCLVKGFYPSDIAVEWESNGQPENNYKTTPPVLDSDGSFFLYSKLTVDKSRWQQGNVFSCSVMHEALHNHYTQKSLSLSPGK

SEQ ID NO: 13 - protein, 369 aa, Artificial Sequence
  Synthetic construct - Unprocessed ActRIIA-hFc with TPA leader sequence
MDAMKRGLCCVLLLCGAVFVSPGAAILGRSETQECLFFNANWEKDRTNQTGVEPCYGDKDKRRHCFATWKNISGSIEIVKQGCWLDDINCYDRTDCVEKKDSPEVYFCCCEGNMCNEKFSYFPEMEVTQPTSNPVTPKPPTGGGTHTCPPCPAPELLGGPSVFLFPPKPKDTLMISRTPEVTCVVVDVSHEDPEVKFNWYVDGVEVHNAKTKPREEQYNSTYRVVSVLTVLHQDWLNGKEYKCKVSNKALPVPIEKTISKAKGQPREPQVYTLPPSREEMTKNQVSLTCLVKGFYPSDIAVEWESNGQPENNYKTTPPVLDSDGSFFLYSKLTVDKSRWQQGNVFSCSVMHEALHNHYTQKSLSLSPGK

SEQ ID NO: 14 - DNA, 1114 bp, Artificial Sequence
  Synthetic construct - Unprocessed ActRIIA-hFc with TPA leader sequence
atggatgcaatgaagagagggctctgctgtgtgctgctgctgtgtggagcagtcttcgtttcgcccggcgccgctatacttggtagatcagaaactcaggagtgtctttttttaatgctaattgggaaaaagacagaaccaatcaaactggtgttgaaccgtgttatggtgacaaagataaacggcggcattgttttgctacctggaagaatatttctggttccattgaatagtgaaacaaggttgttggctggatgatatcaactgctatgacaggactgattgtgtagaaaaaaaagacagccctgaagtatatttctgttgctgtgagggcaatatgtgtaatgaaaagttttcttattttccggagatggaagtcacacagcccacttcaaatccagttacacctaagccacccaccggtggtggaactcacacatgcccaccgtgcccagcacctgaactcctggggggaccgtcagtcttcctcttccccccaaaacccaaggacaccctcatgatctcccggacccctgaggtcacatgcgtggtggtggacgtgagccacgaagaccctgaggtcaagttcaactggtacgtggacggcgtggaggtgcataatgccaagacaaagccgcgggaggagcagtacaacagcacgtaccgtgtggtcagcgtcctcaccgtcctgcaccaggactggctgaatggcaaggagtacaagtgcaaggtctccaacaaagccctcccagtccccatcgagaaaaccatctccaaagccaaagggcagccccgagaaccacaggtgtacaccctgcccccatcccgggaggagatgaccaagaaccaggtcagcctgacctgcctggtcaaaggcttctatcccagcgacatcgccgtggagtgggagagcaatgggcagccggagaacaactacaagaccacgcctcccgtgctggactccgacggctccttcttcctctatagcaagctcaccgtggacaagagcaggtggcagcaggggaacgtcttctcatgctccgtgatgcatgaggctctgcacaaccactacacgcagaagagcctctccctgtctccgggtaaatgagaattc

SEQ ID NO: 15 - protein, 106 aa, Artificial Sequence
  Synthetic construct - human ActRIIB soluble (extracellular), processed polypeptide sequence with the N-terminal 6 amino acid of the EC domain deleted and the C-terminal 4 amino acids of the EC domain deleted
ETRECIYYNANWELERTNQSGLERCEGEQDKRLHCYASWRNSSGTIELVKKGCWDDDFNCYDRQECVATEENPQVYFCCCEGNFCNERFTHLPEAGGPEVTYEPPP

SEQ ID NO: 16 - protein, 512 aa, Homo sapiens
  human ActRIIB precursor protein
MTAPWVALALLWGSLWPGSGRGEAETRECIYYNANWELERTNQSGLERCEGEQDKRLHCYASWANSSGTIELVKKGCWLDDFNCYDRQECVATEENPQVYFCCCEGNFCNERFTHLPEAGGPEVTYEPPPTAPTLLTVLAYSLLPIGGLSLIVLLAFWMYRHRKPPYGHVDIHEDPGPPPPSPLVGLKPLQLLEIKARGRFGCVWKAQLMNDFVAVKIFPLQDKQSWQSEREIFSTPGMKHENLLQFIAAEKRGSNLEVELWLITAFHDKGSLTDYLKGNIITWNELCHVAETMSRGLSYLHEDVPWCRGEGHKPSIAHRDFKSKNVLLKSDLTAVLADFGLAVRFEPGKPPGDTHGQVGTRRYMAPEVLEGAINFQRDAFLRIDMYAMGLVLWELVSRCKAADGPVDEYMLPFEEEIGQHPSLEELQEVVVHKKMRPTIKDHWLKHPGLAQLCVTIEECWDHDAEARLSAGCVEERVSLIRRSVNGTTSDCLVSLVTSVTNVDLPPKESSI

SEQ ID NO: 17 - protein, 116 aa, Homo sapiens
  human ActRIIB soluble (extracellular), processed polypeptide
SGRGEAETRECIYYNANWELERTNQSGLERCEGEQDKRLHCYASWANSSGTIELVKKGCWLDDFNCYDRQECVATEENPQVYFCCCEGNFCNERFTHLPEAGGPEVTYEPPPTAPT

SEQ ID NO: 18 - protein, 101 aa, Artificial Sequence
  human ActRIIB soluble (extracellular), processed polypeptide sequence with the C-terminal 15 amino acids deleted
SGRGEAETRECIYYNANWELERTNQSGLERCEGEQDKRLHCYASWANSSGTIELVKKGCWLDDFNCYDRQECVATEENPQVYFCCCEGNFCNERFTHLPEA

SEQ ID NO: 19 - DNA, 1539 bp, Homo sapiens
  human ActRIIB (A64) precursor
atgacggcgccctgggtggccctcgccctcctctggggatcgctgtggcccggctctgggcgtggggaggctgagacacgggagtgcatctactacaacgccaactgggagctggagcgcaccaaccagagcggcctggagcgctgcgaaggcgagcaggacaagcggctgcactgctacgcctcctgggccaacagctctggcaccatcgagctcgtgaagaagggctgctggctagatgacttcaactgctacgataggcaggagtgtgtggccactgaggagaacccccaggtgtacttctgctgctgtgaaggcaacttctgcaacgagcgcttcactcatttgccagaggctgggggcccggaagtcacgtacgagccacccccgacagcccccaccctgctcacggtgctggcctactcactgctgcccatcgggggcctttccctcatcgtcctgctggccttttggatgtaccggcatcgcaagcccccctacggtcatgtggacatccatgaggaccctgggcctccaccaccatcccctctggtgggcctgaagccactgcagctgctggagatcaaggctcgggggcgctttggctgtgtctggaaggcccagctcatgaatgactttgtagctgtcaagatcttcccactccaggacaagcagtcgtggcagagtgaacgggagatcttcagcacacctggcatgaagcacgagaacctgctacagttcattgctgccgagaagcgaggctccaacctcgaagtagagctgtggctcatcacggccttccatgacaagggctccctcacggattacctcaaggggaacatcatcacatggaacgaactgtgtcatgtagcagagacgatgtcacgaggcctctcatacctgcatgaggatgtgccctggtgccgtggcgagggccacaagccgtctattgcccacagggactttaaaagtaagaatgtattgctgaagagcgacctcacagccgtgctggctgactttggcttggctgttcgatttgagccagggaaacctccaggggacacccacggacaggtaggcacgagacggtacatggctcctgaggtgctcgagggagccatcaacttccagagagatgccttcctgcgcattgacatgtatgccatggggttggtgctgtgggagcttgtgtctcgctgcaaggctgcagacggacccgtggatgagtacatgctgccctttgaggaagagattggccagcacccttcgttggaggagctgcaggaggtggtggtgcacaagaagatgaggcccaccattaaagatcactggttgaaacacccgggcctggcccagctttgtgtgaccatcgaggagtgctgggaccatgatgcagaggctcgcttgtccgcgggctgtgtggaggagcgggtgtccctgattcggaggtcggtcaacggcactacctcggactgtctcgtttccctggtgacctctgtcaccaatgtggacctgccccctaaagagtcaagcatctaa

SEQ ID NO: 20 - protein, 344 aa, Artificial Sequence
  Synthetic construct - fusion protein comprising a soluble extracellular domain of ActRIIB fused to an Fc domain
SGRGEAETRECIYYNANWELERTNQSGLERCEGEQDKRLHCYASWANSSGTIELVKKGCWLDDFNCYDRQECVATEENPQVYFCCCEGNFCNERFTHLPEAGGPEVTYEPPPTAPTGGGTHTCPPCPAPELLGGPSVFLFPPKPKDTLMISRTPEVTCVVVDVSHEDPEVKFNWYVDGVEVHNAKTKPREEQYNSTYRVVSVLTVLHQDWLNGKEYKCKVSNKALPVPIEKTISKAKGQPREPQVYTLPPSREEMTKNQVSLTCLVKGFYPSDIAVEWESNGQPENNYKTTPPVLDSDGSFFLYSKLTVDKSRWQQGNVFSCSVMHEALHNHYTQKSLSLSPGK

SEQ ID NO: 21 - protein, 329 aa, Artificial Sequence
  Synthetic construct - fusion protein comprising a soluble extracellular domain of ActRIIB (A64) with the C-terminal 15 amino acids deleted fused to an Fc domain
SGRGEAETRECIYYNANWELERTNQSGLERCEGEQDKRLHCYASWANSSGTIELVKKGCWLDDFNCYDRQECVATEENPQVYFCCCEGNFCNERFTHLPEAGGGTHTCPPCPAPELLGGPSVFLFPPKPKDTLMISRTPEVTCVVVDVSHEDPEVKFNWYVDGVEVHNAKTKPREEQYNSTYRVVSVLTVLHQDWLNGKEYKCKVSNKALPVPIEKTISKAKGQPREPQVYTLPPSREEMTKNQVSLTCLVKGFYPSDIAVEWESNGQPENNYKTTPPVLDSDGSFFLYSKLTVDKSRWQQGNVFSCSVMHEALHNHYTQKSLSLSPGK

SEQ ID NO: 22 - protein, 105 aa, Artificial Sequence
  human ActRIIB soluble (extracellular), processed polypeptide with the N-terminal 6 amino acids of the EC domain deleted and the C-terminal 5 amino acids of the EC domain deleted and with an L79D mutation
ETRECIYYNANWELERTNQSGLERCEGEQDKRLHCYASWRNSSGTIELVKKGCWDDDFNCYDRQECVATEENPQVYFCCCEGNFCNERFTHLPEAGGPEVTYEPP

SEQ ID NO: 23 - protein, 107 aa, Artificial Sequence
  human ActRIIB soluble (extracellular), processed polypeptide sequence with the N-terminal 6 amino acids of the EC domain deleted and the C-terminal 3 amino acids of the EC domain deleted and with an L79D mutatioN
ETRECIYYNANWELERTNQSGLERCEGEQDKRLHCYASWRNSSGTIELVKKGCWDDDFNCYDRQECVATEENPQVYFCCCEGNFCNERFTHLPEAGGPEVTYEPPPT

SEQ ID NO: 24 - protein, 360 aa, Artificial Sequence
  Unprocessed ActRIIB-Fc fusion protein with the N-terminal 6 amino acids of the EC domain deleted and the C-terminal 3 amino acids of the EC domain deleted and with an L79D mutation and with TPA leader sequence
MDAMKRGLCCVLLLCGAVFVSPGAAETRECIYYNANWELERTNQSGLERCEGEQDKRLHCYASWRNSSGTIELVKKGCWDDDFNCYDRQECVATEENPQVYFCCCEGNFCNERFTHLPEAGGPEVTYEPPPTGGGTHTCPPCPAPELLGGPSVFLFPPKPKDTLMISRTPEVTCVVVDVSHEDPEVKFNWYVDGVEVHNAKTKPREEQYNSTYRVVSVLTVLHQDWLNGKEYKCKVSNKALPAPIEKTISKAKGQPREPQVYTLPPSREEMTKNQVSLTCLVKGFYPSDIAVEWESNGQPENNYKTTPPVLDSDGSFFLYSKLTVDKSRWQQGNVFSCSVMHEALHNHYTQKSLSLSPGK

SEQ ID NO: 25 - protein, 335 aa, Artificial Sequence
  Processed ActRIIB-Fc fusion protein with the N-terminal 6 amino acids of the EC domain deleted and the C-terminal 3 amino acids of the EC domain deleted and with an L79D mutation
ETRECIYYNANWELERTNQSGLERCEGEQDKRLHCYASWRNSSGTIELVKKGCWDDDFNCYDRQECVATEENPQVYFCCCEGNFCNERFTHLPEAGGPEVTYEPPPTGGGTHTCPPCPAPELLGGPSVFLFPPKPKDTLMISRTPEVTCVVVDVSHEDPEVKFNWYVDGVEVHNAKTKPREEQYNSTYRVVSVLTVLHQDWLNGKEYKCKVSNKALPAPIEKTISKAKGQPREPQVYTLPPSREEMTKNQVSLTCLVKGFYPSDIAVEWESNGQPENNYKTTPPVLDSDGSFFLYSKLTVDKSRWQQGNVFSCSVMHEALHNHYTQKSLSLSPGK

SEQ ID NO: 26 - protein, 115 aa, Homo sapiens
  human ActRIIB soluble (extracellular) processed polypeptide
GRGEAETRECIYYNANWELERTNQSGLERCEGEQDKRLHCYASWANSSGTIELVKKGCWLDDFNCYDRQECVATEENPQVYFCCCEGNFCNERFTHLPEAGGPEVTYEPPPTAPT

SEQ ID NO: 27 - protein, 100 aa, Artificial Sequence
  human ActRIIB soluble (extracellular) processed polypeptide sequence with the C-terminal 15 amino acids deleted
GRGEAETRECIYYNANWELERTNQSGLERCEGEQDKRLHCYASWANSSGTIELVKKGCWLDDFNCYDRQECVATEENPQVYFCCCEGNFCNERFTHLPEA

SEQ ID NO: 28 - protein, 512 aa, Homo sapiens
  human ActRIIB precursor protein
MTAPWVALALLWGSLWPGSGRGEAETRECIYYNANWELERTNQSGLERCEGEQDKRLHCYASWRNSSGTIELVKKGCWLDDFNCYDRQECVATEENPQVYFCCCEGNFCNERFTHLPEAGGPEVTYEPPPTAPTLLTVLAYSLLPIGGLSLIVLLAFWMYRHRKPPYGHVDIHEDPGPPPPSPLVGLKPLQLLEIKARGRFGCVWKAQLMNDFVAVKIFPLQDKQSWQSEREIFSTPGMKHENLLQFIAAEKRGSNLEVELWLITAFHDKGSLTDYLKGNIITWNELCHVAETMSRGLSYLHEDVPWCRGEGHKPSIAHRDFKSKNVLLKSDLTAVLADFGLAVRFEPGKPPGDTHGQVGTRRYMAPEVLEGAINFQRDAFLRIDMYAMGLVLWELVSRCKAADGPVDEYMLPFEEEIGQHPSLEELQEVVVHKKMRPTIKDHWLKHPGLAQLCVTIEECWDHDAEARLSAGCVEERVSLIRRSVNGTTSDCLVSLVTSVTNVDLPPKESSI

SEQ ID NO: 29 - protein, 116 aa, Homo sapiens
  human ActRIIB soluble (extracellular) processed polypeptide
SGRGEAETRECIYYNANWELERTNQSGLERCEGEQDKRLHCYASWRNSSGTIELVKKGCWLDDFNCYDRQECVATEENPQVYFCCCEGNFCNERFTHLPEAGGPEVTYEPPPTAPT

SEQ ID NO: 30 - protein, 101 aa, Artificial Sequence
  human ActRIIB soluble (extracellular), processed polypeptide with the C-terminal 15 amino acids deleted
SGRGEAETRECIYYNANWELERTNQSGLERCEGEQDKRLHCYASWRNSSGTIELVKKGCWLDDFNCYDRQECVATEENPQVYFCCCEGNFCNERFTHLPEA

SEQ ID NO: 31 - protein, 115 aa, Homo sapiens
  human ActRIIB soluble (extracellular), processed polypeptide
GRGEAETRECIYYNANWELERTNQSGLERCEGEQDKRLHCYASWRNSSGTIELVKKGCWLDDFNCYDRQECVATEENPQVYFCCCEGNFCNERFTHLPEAGGPEVTYEPPPTAPT

SEQ ID NO: 32 - protein, 100 aa, Artificial Sequence
  human ActRIIB soluble (extracellular), processed polypeptide with the C-terminal 15 amino acids deleted
GRGEAETRECIYYNANWELERTNQSGLERCEGEQDKRLHCYASWRNSSGTIELVKKGCWLDDFNCYDRQECVATEENPQVYFCCCEGNFCNERFTHLPEA

SEQ ID NO: 33 - protein, 107 aa, Artificial Sequence
  human ActRIIB soluble (extracellular), processed polypeptide sequence with the N-terminal 6 amino acids of the EC domain deleted and the C-terminal 3 amino acids of the EC domain deleted and with an L79D mutation
ETRECIYYNANWELERTNQSGLERCEGEQDKRLHCYASWANSSGTIELVKKGCWDDDFNCYDRQECVATEENPQVYFCCCEGNFCNERFTHLPEAGGPEVTYEPPPT

SEQ ID NO: 34 - protein, 360 aa, Artificial Sequence
  Unprocessed ActRIIB-Fc fusion protein with the N-terminal 6 amino acids of the EC domain deleted and the C-terminal 3 amino acids of the EC domain deleted and with an L79D mutation and with TPA leader sequence
MDAMKRGLCCVLLLCGAVFVSPGAAETRECIYYNANWELERTNQSGLERCEGEQDKRLHCYASWANSSGTIELVKKGCWDDDFNCYDRQECVATEENPQVYFCCCEGNFCNERFTHLPEAGGPEVTYEPPPTGGGTHTCPPCPAPELLGGPSVFLFPPKPKDTLMISRTPEVTCVVVDVSHEDPEVKFNWYVDGVEVHNAKTKPREEQYNSTYRVVSVLTVLHQDWLNGKEYKCKVSNKALPAPIEKTISKAKGQPREPQVYTLPPSREEMTKNQVSLTCLVKGFYPSDIAVEWESNGQPENNYKTTPPVLDSDGSFFLYSKLTVDKSRWQQGNVFSCSVMHEALHNHYTQKSLSLSPGK

SEQ ID NO: 35 - protein, 335 aa, Artificial Sequence
  Processed ActRIIB-Fc fusion protein with the N-terminal 6 amino acids of the EC domain deleted and the C-terminal 3 amino acids of the EC domain deleted and with an L79D mutation
ETRECIYYNANWELERTNQSGLERCEGEQDKRLHCYASWANSSGTIELVKKGCWDDDFNCYDRQECVATEENPQVYFCCCEGNFCNERFTHLPEAGGPEVTYEPPPTGGGTHTCPPCPAPELLGGPSVFLFPPKPKDTLMISRTPEVTCVVVDVSHEDPEVKFNWYVDGVEVHNAKTKPREEQYNSTYRVVSVLTVLHQDWLNGKEYKCKVSNKALPAPIEKTISKAKGQPREPQVYTLPPSREEMTKNQVSLTCLVKGFYPSDIAVEWESNGQPENNYKTTPPVLDSDGSFFLYSKLTVDKSRWQQGNVFSCSVMHEALHNHYTQKSLSLSPGK

SEQ ID NO: 36 - protein, 115 aa, Artificial Sequence
  human ActRIIB soluble (extracellular), processed polypeptide sequence with L79D mutation
GRGEAETRECIYYNANWELERTNQSGLERCEGEQDKRLHCYASWRNSSGTIELVKKGCWDDDFNCYDRQECVATEENPQVYFCCCEGNFCNERFTHLPEAGGPEVTYEPPPTAPT

SEQ ID NO: 37 - protein, 115 aa, Artificial Sequence
  human ActRIIB soluble (extracellular), processed polypeptide sequence with L79D mutation
GRGEAETRECIYYNANWELERTNQSGLERCEGEQDKRLHCYASWANSSGTIELVKKGCWDDDFNCYDRQECVATEENPQVYFCCCEGNFCNERFTHLPEAGGPEVTYEPPPTAPT

SEQ ID NO: 38 - protein, 343 aa, Artificial Sequence
  human ActRIIB soluble (extracellular), processed polypeptide sequence with L79D mutation fused to an Fc domain with a GGG linker
GRGEAETRECIYYNANWELERTNQSGLERCEGEQDKRLHCYASWRNSSGTIELVKKGCWDDDFNCYDRQECVATEENPQVYFCCCEGNFCNERFTHLPEAGGPEVTYEPPPTAPTGGGTHTCPPCPAPELLGGPSVFLFPPKPKDTLMISRTPEVTCVVVDVSHEDPEVKFNWYVDGVEVHNAKTKPREEQYNSTYRVVSVLTVLHQDWLNGKEYKCKVSNKALPAPIEKTISKAKGQPREPQVYTLPPSREEMTKNQVSLTCLVKGFYPSDIAVEWESNGQPENNYKTTPPVLDSDGSFFLYSKLTVDKSRWQQGNVFSCSVMHEALHNHYTQKSLSLSPGK

SEQ ID NO: 39 - protein, 343 aa, Artificial Sequence
  human ActRIIB soluble (extracellular), processed polypeptide sequence with L79D mutation fused to an Fc domain
GRGEAETRECIYYNANWELERTNQSGLERCEGEQDKRLHCYASWANSSGTIELVKKGCWDDDFNCYDRQECVATEENPQVYFCCCEGNFCNERFTHLPEAGGPEVTYEPPPTAPTGGGTHTCPPCPAPELLGGPSVFLFPPKPKDTLMISRTPEVTCVVVDVSHEDPEVKFNWYVDGVEVHNAKTKPREEQYNSTYRVVSVLTVLHQDWLNGKEYKCKVSNKALPAPIEKTISKAKGQPREPQVYTLPPSREEMTKNQVSLTCLVKGFYPSDIAVEWESNGQPENNYKTTPPVLDSDGSFFLYSKLTVDKSRWQQGNVFSCSVMHEALHNHYTQKSLSLSPGK

SEQ ID NO: 40 - protein, 368 aa, Artificial Sequence
  human ActRIIB soluble (extracellular), processed polypeptide sequence with L79D mutation fused to an Fc domain and with TPA leader sequence
MDAMKRGLCCVLLLCGAVFVSPGASGRGEAETRECIYYNANWELERTNQSGLERCEGEQDKRLHCYASWRNSSGTIELVKKGCWDDDFNCYDRQECVATEENPQVYFCCCEGNFCNERFTHLPEAGGPEVTYEPPPTAPTGGGTHTCPPCPAPELLGGPSVFLFPPKPKDTLMISRTPEVTCVVVDVSHEDPEVKFNWYVDGVEVHNAKTKPREEQYNSTYRVVSVLTVLHQDWLNGKEYKCKVSNKALPAPIEKTISKAKGQPREPQVYTLPPSREEMTKNQVSLTCLVKGFYPSDIAVEWESNGQPENNYKTTPPVLDSDGSFFLYSKLTVDKSRWQQGNVFSCSVMHEALHNHYTQKSLSLSPGK

SEQ ID NO: 41 - protein, 368 aa, Artificial Sequence
  human ActRIIB soluble (extracellular), processed polypeptide sequence with L79D mutation fused to an Fc domain and with TPA leader sequence
MDAMKRGLCCVLLLCGAVFVSPGASGRGEAETRECIYYNANWELERTNQSGLERCEGEQDKRLHCYASWANSSGTIELVKKGCWDDDFNCYDRQECVATEENPQVYFCCCEGNFCNERFTHLPEAGGPEVTYEPPPTAPTGGGTHTCPPCPAPELLGGPSVFLFPPKPKDTLMISRTPEVTCVVVDVSHEDPEVKFNWYVDGVEVHNAKTKPREEQYNSTYRVVSVLTVLHQDWLNGKEYKCKVSNKALPAPIEKTISKAKGQPREPQVYTLPPSREEMTKNQVSLTCLVKGFYPSDIAVEWESNGQPENNYKTTPPVLDSDGSFFLYSKLTVDKSRWQQGNVFSCSVMHEALHNHYTQKSLSLSPGK

SEQ ID NO: 42 - protein, 141 aa, Artificial Sequence
  human ActRIIB soluble (extracellular), processed polypeptide having a variant C-terminal sequence
GRGEAETRECIYYNANWELERTNQSGLERCEGEQDKRLHCYASWRNSSGTIELVKKGCWLDDFNCYDRQECVATEENPQVYFCCCEGNFCNERFTHLPEAGGPEGPWASTTIPSGGPEATAAAGDQGSGALWLCLEGPAHE

SEQ ID NO: 43 - protein, 141 aa, Artificial Sequence
  human ActRIIB soluble (extracellular), processed polypeptide having a variant C-terminal sequence having an L79D mutation
GRGEAETRECIYYNANWELERTNQSGLERCEGEQDKRLHCYASWRNSSGTIELVKKGCWDDDFNCYDRQECVATEENPQVYFCCCEGNFCNERFTHLPEAGGPEGPWASTTIPSGGPEATAAAGDQGSGALWLCLEGPAHE

SEQ ID NO: 44 - protein, 370 aa, Artificial Sequence
  human ActRIIB soluble (extracellular), processed polypeptide sequence having a variant C-terminal sequence having an L79D mutation fused to an Fc domain with a TGGG linker
GRGEAETRECIYYNANWELERTNQSGLERCEGEQDKRLHCYASWRNSSGTIELVKKGCWDDDFNCYDRQECVATEENPQVYFCCCEGNFCNERFTHLPEAGGPEGPWASTTIPSGGPEATAAAGDQGSGALWLCLEGPAHETGGGTHTCPPCPAPELLGGPSVFLFPPKPKDTLMISRTPEVTCVVVDVSHEDPEVKFNWYVDGVEVHNAKTKPREEQYNSTYRVVSVLTVLHQDWLNGKEYKCKVSNKALPAPIEKTISKAKGQPREPQVYTLPPSREEMTKNQVSLTCLVKGFYPSDIAVEWESNGQPENNYKTTPPVLDSDGSFFLYSKLTVDKSRWQQGNVFSCSVMHEALHNHYTQKSLSLSPGK

SEQ ID NO: 45 - DNA, 1083 bp, Artificial Sequence
  Unprocessed ActRIIB-Fc fusion protein with the N-terminal 6 amino acids of the EC domain deleted and the C-terminal 3 amino acids of the EC domain deleted and with an L79D mutation and with TPA leader sequence
atggatgcaatgaagagagggctctgctgtgtgctgctgctgtgtggagcagtcttcgtttcgcccggcgccgccgaaacccgcgaatgtatttattacaatgctaattgggaactcgaacggacgaaccaatccgggctcgaacggtgtgagggggaacaggataaacgcctccattgctatgcgtcgtggaggaactcctccgggacgattgaactggtcaagaaagggtgctgggacgacgatttcaattgttatgaccgccaggaatgtgtcgcgaccgaagagaatccgcaggtctatttctgttgttgcgaggggaatttctgtaatgaacggtttacccacctccccgaagccggcgggcccgaggtgacctatgaacccccgcccaccggtggtggaactcacacatgcccaccgtgcccagcacctgaactcctggggggaccgtcagtcttcctcttccccccaaaacccaaggacaccctcatgatctcccggacccctgaggtcacatgcgtggtggtggacgtgagccacgaagaccctgaggtcaagttcaactggtacgtggacggcgtggaggtgcataatgccaagacaaagccgcgggaggagcagtacaacagcacgtaccgtgtggtcagcgtcctcaccgtcctgcaccaggactggctgaatggcaaggagtacaagtgcaaggtctccaacaaagccctcccagcccccatcgagaaaaccatctccaaagccaaagggcagccccgagaaccacaggtgtacaccctgcccccatcccgggaggagatgaccaagaaccaggtcagcctgacctgcctggtcaaaggcttctatcccagcgacatcgccgtggagtgggagagcaatgggcagccggagaacaactacaagaccacgcctcccgtgctggactccgacggctccttcttcctctatagcaagctcaccgtggacaagagcaggtggcagcaggggaacgtcttctcatgctccgtgatgcatgaggctctgcacaaccactacacgcagaagagcctctccctgtccccgggtaaatga

SEQ ID NO: 46 - protein, 344 aa, Artificial Sequence
  fusion protein comprising a soluble extracellular domain of ActRIIB fused to an Fc domain
SGRGEAETRECIYYNANWELERTNQSGLERCEGEQDKRLHCYASWRNSSGTIELVKKGCWLDDFNCYDRQECVATEENPQVYFCCCEGNFCNERFTHLPEAGGPEVTYEPPPTAPTGGGTHTCPPCPAPELLGGPSVFLFPPKPKDTLMISRTPEVTCVVVDVSHEDPEVKFNWYVDGVEVHNAKTKPREEQYNSTYRVVSVLTVLHQDWLNGKEYKCKVSNKALPVPIEKTISKAKGQPREPQVYTLPPSREEMTKNQVSLTCLVKGFYPSDIAVEWESNGQPENNYKTTPPVLDSDGSFFLYSKLTVDKSRWQQGNVFSCSVMHEALHNHYTQKSLSLSPGK

SEQ ID NO: 47 - protein, 329 aa, Artificial Sequence
  fusion protein comprising a soluble extracellular domain of ActRIIB (R64) with the C-terminal 15 amino acids deleted fused to an Fc domain
SGRGEAETRECIYYNANWELERTNQSGLERCEGEQDKRLHCYASWRNSSGTIELVKKGCWLDDFNCYDRQECVATEENPQVYFCCCEGNFCNERFTHLPEAGGGTHTCPPCPAPELLGGPSVFLFPPKPKDTLMISRTPEVTCVVVDVSHEDPEVKFNWYVDGVEVHNAKTKPREEQYNSTYRVVSVLTVLHQDWLNGKEYKCKVSNKALPVPIEKTISKAKGQPREPQVYTLPPSREEMTKNQVSLTCLVKGFYPSDIAVEWESNGQPENNYKTTPPVLDSDGSFFLYSKLTVDKSRWQQGNVFSCSVMHEALHNHYTQKSLSLSPGK

SEQ ID NO: 48 - protein, 407 aa, Unknown
  full-length, unprocessed precursor protein GDF11 (GDF11 preproprotein)
MVLAAPLLLGFLLLALELRPRGEAAEGPAAAAAAAAAAAAAGVGGERSSRPAPSVAPEPDGCPVCVWRQHSRELRLESIKSQILSKLRLKEAPNISREVVKQLLPKAPPLQQILDLHDFQGDALQPEDFLEEDEYHATTETVISMAQETDPAVQTDGSPLCCHFHFSPKVMFTKVLKAQLWVYLRPVPRPATVYLQILRLKPLTGEGTAGGGGGGRRHIRIRSLKIELHSRSGHWQSIDFKQVLHSWFRQPQSNWGIEINAFDPSGTDLAVTSLGPGAEGLHPFMELRVLENTKRSRRNLGLDCDEHSSESRCCRYPLTVDFEAFGWDWIIAPKRYKANYCSGQCEYMFMQKYPHTHLVQQANPRGSAGPCCTPTKMSPINMLYFNDKQQIIYGKIPGMVVDRCGCS

SEQ ID NO: 49 - DNA, 1221 bp, Unknown
  full-length, unprocessed precursor protein GDF11 (GDF11 preproprotein)
atggtgctcgcggccccgctgctgctgggcttcctgctcctcgccctggagctgcggccccggggggaggcggccgagggccccgcggcggcggcggcggcggcggcggcggcggcagcggcgggggtcgggggggagcgctccagccggccagccccgtccgtggcgcccgagccggacggctgccccgtgtgcgtttggcggcagcacagccgcgagctgcgcctagagagcatcaagtcgcagatcttgagcaaactgcggctcaaggaggcgcccaacatcagccgcgaggtggtgaagcagctgctgcccaaggcgccgccgctgcagcagatcctggacctacacgacttccagggcgacgcgctgcagcccgaggacttcctggaggaggacgagtaccacgccaccaccgagaccgtcattagcatggcccaggagacggacccagcagtacagacagatggcagccctctctgctgccattttcacttcagccccaaggtgatgttcacaaaggtactgaaggcccagctgtgggtgtacctacggcctgtaccccgcccagccacagtctacctgcagatcttgcgactaaaacccctaactggggaagggaccgcagggggagggggcggaggccggcgtcacatccgtatccgctcactgaagattgagctgcactcacgctcaggccattggcagagcatcgacttcaagcaagtgctacacagctggttccgccagccacagagcaactggggcatcgagatcaacgcctttgatcccagtggcacagacctggctgtcacctccctggggccgggagccgaggggctgcatccattcatggagcttcgagtcctagagaacacaaaacgttcccggcggaacctgggtctggactgcgacgagcactcaagcgagtcccgctgctgccgatatcccctcacagtggactttgaggctttcggctgggactggatcatcgcacctaagcgctacaaggccaactactgctccggccagtgcgagtacatgttcatgcaaaaatatccgcatacccatttggtgcagcaggccaatccaagaggctctgctgggccctgttgtacccccaccaagatgtccccaatcaacatgctctacttcaatgacaagcagcagattatctacggcaagatccctggcatggtggtggatcgctgtggctgctct

SEQ ID NO: 50 - protein, 274 aa, Homo sapiens
  GDF11 propeptide of human GDF11 protein
AEGPAAAAAAAAAAAAAGVGGERSSRPAPSVAPEPDGCPVCVWRQHSRELRLESIKSQILSKLRLKEAPNISREVVKQLLPKAPPLQQILDLHDFQGDALQPEDFLEEDEYHATTETVISMAQETDPAVQTDGSPLCCHFHFSPKVMFTKVLKAQLWVYLRPVPRPATVYLQILRLKPLTGEGTAGGGGGGRRHIRIRSLKIELHSRSGHWQSIDFKQVLHSWFRQPQSNWGIEINAFDPSGTDLAVTSLGPGAEGLHPFMELRVLENTKRSRR

SEQ ID NO: 51 - DNA, 822 bp, Homo sapiens
  GDF11 propeptide of human GDF11 protein
gccgagggccccgcggcggcggcggcggcggcggcggcggcggcagcggcgggggtcgggggggagcgctccagccggccagccccgtccgtggcgcccgagccggacggctgccccgtgtgcgtttggcggcagcacagccgcgagctgcgcctagagagcatcaagtcgcagatcttgagcaaactgcggctcaaggaggcgcccaacatcagccgcgaggtggtgaagcagctgctgcccaaggcgccgccgctgcagcagatcctggacctacacgacttccagggcgacgcgctgcagcccgaggacttcctggaggaggacgagtaccacgccaccaccgagaccgtcattagcatggcccaggagacggacccagcagtacagacagatggcagccctctctgctgccattttcacttcagccccaaggtgatgttcacaaaggtactgaaggcccagctgtgggtgtacctacggcctgtaccccgcccagccacagtctacctgcagatcttgcgactaaaacccctaactggggaagggaccgcagggggagggggcggaggccggcgtcacatccgtatccgctcactgaagattgagctgcactcacgctcaggccattggcagagcatcgacttcaagcaagtgctacacagctggttccgccagccacagagcaactggggcatcgagatcaacgcctttgatcccagtggcacagacctggctgtcacctccctggggccgggagccgaggggctgcatccattcatggagcttcgagtcctagagaacacaaaacgttcccggcgg

SEQ ID NO: 52 - protein, 109 aa, Homo sapiens
  Mature human GDF11 protein
NLGLDCDEHSSESRCCRYPLTVDFEAFGWDWIIAPKRYKANYCSGQCEYMFMQKYPHTHLVQQANPRGSAGPCCTPTKMSPINMLYFNDKQQIIYGKIPGMVVDRCGCS

SEQ ID NO: 53 - DNA, 327 bp, Homo sapiens
  GDF11 propeptide of human GDF11 protein
aacctgggtctggactgcgacgagcactcaagcgagtcccgctgctgccgatatcccctcacagtggactttgaggctttcggctgggactggatcatcgcacctaagcgctacaaggccaactactgctccggccagtgcgagtacatgttcatgcaaaaatatccgcatacccatttggtgcagcaggccaatccaagaggctctgctgggccctgttgtacccccaccaagatgtccccaatcaacatgctctacttcaatgacaagcagcagattatctacggcaagatccctggcatggtggtggatcgctgtggctgctct